European Patent Application EP 4 166 565 A1, published April 19, 2023. Title: Method for producing dipeptide. Applicant: KYOWA HAKKO BIO CO., LTD. The sequence listing filed with the application follows.

SEQUENCE LISTING (119 sequences)

SEQ ID NO: 1 - DNA, 1419 bp, Bacillus subtilis
atggagagaaaaacagtattggtcatcgctgatcttggaggctgcccgccgcacatgttttataaaagcgctgctgaaaaatataacctggtcagctttattccaagaccttttgcaattacagcctcccatgcagcattgattgaaaaatactcggtcgcggtcataaaagataaagactattttaagagtttagctgattttgaacaccctgattccatttattgggcgcatgaagatcataacaagcctgaggaagaggtcgtcgagcaaatcgtcaaggttgccgaaatgtttggggcggatgccatcacaacaaacaatgaattattcattgctccgatggcgaaagcctgtgaacgtctgggcttgagaggtgccggcgtgcaggcagccgaaaatgccagagataaaaataaaatgagggacgcttttaataaggccggagtcaaatcgatcaaaaacaaacgagtcacaactcttgaagatttccgtgctgctcttgaagagatcggcacacctcttatcttaaagcctacatacttagcgagttctatcggtgtaacgctgattacggacactgagacggcagaagatgaatttaacagagtcaatgactatctgaaatcaattaacgtgccaaaggcggttacgtttgaagcgccgtttatcgctgaagaatttttacagggtgagtacggagactggtatcaaacagaagggtactccgactatatcagtatagaaggcatcatggctgacggtgagtatttcccgatcgccattcatgataaaacgccgcaaatcgggtttacagagacatcccacattacgccgtccattctggatgaagaggcaaaaaagaaaattgtcgaagctgccaaaaaggcaaatgaagggcttggactgcaaaattgcgcaacacatacagagatcaagctaatgaaaaacagagaaccgggtttaatagagtcggcagccagatttgccggctggaatatgatccccaatattaaaaaggtctttggccttgatatggcgcaattattattagatgtcctctgtttcggaaaagacgccgatctgccggacggattattggatcaagagccttattatgttgccgactgccatttgtacccgcagcatttcaaacaaaatggccaaattcctgaaactgctgaggatttggtcattgaagcgatcgatattccggacgggcttttaaaaggggatactgaaatcgtttctttttcggccgcagcaccaggcacttcagttgatttgacattgtttgaagctttcaattccattgctgcatttgaactgaaaggcagtaattcacaggatgtggctgaatcaatcagacaaattcagcagcatgcgaagctgacggcaaagtatgtgctgccagtatga

SEQ ID NO: 2 - protein, 472 aa, Bacillus subtilis
MERKTVLVIADLGGCPPHMFYKSAAEKYNLVSFIPRPFAITASHAALIEKYSVAVIKDKDYFKSLADFEHPDSIYWAHEDHNKPEEEVVEQIVKVAEMFGADAITTNNELFIAPMAKACERLGLRGAGVQAAENARDKNKMRDAFNKAGVKSIKNKRVTTLEDFRAALEEIGTPLILKPTYLASSIGVTLITDTETAEDEFNRVNDYLKSINVPKAVTFEAPFIAEEFLQGEYGDWYQTEGYSDYISIEGIMADGEYFPIAIHDKTPQIGFTETSHITPSILDEEAKKKIVEAAKKANEGLGLQNCATHTEIKLMKNREPGLIESAARFAGWNMIPNIKKVFGLDMAQLLLDVLCFGKDADLPDGLLDQEPYYVADCHLYPQHFKQNGQIPETAEDLVIEAIDIPDGLLKGDTEIVSFSAAAPGTSVDLTLFEAFNSIAAFELKGSNSQDVAESIRQIQQHAKLTAKYVLPV

SEQ ID NO: 3 - protein, 472 aa, Bacillus amyloliquefaciens
MERKTVLVIADLGGCPPHMFYESAAEKYNLVSFIPRPFAITASHAALIEKYSIAVIKDKDYFKSLADFEHPDSIYWAHEDHDKPEEEVVEEIVKVADMFAVDAITTNNELFIAPMAKACKRLGLRGAGVQAAENARDKNKMRAAFNRAGVKSIKNKRVTTLEDFRAALQEIGTPLILKPTYLASSIGVTLIKEMETAEAEFNRVNEYLKSINVPKAVTFEAPFIAEEFLQGEYDDWYETSGYSDYISIEGIMADGEYFPVAIHDKTPQIGFTETAHITPSILDDDAKRKIVEAAKKANEGLGLENCATHTEIKLMKNREAGLIESAPRFAGWNMIPNIKKVFGVDMAQLLLDVLCFGKEADLPKGLLEQEPCYVADCHLYPQHFKENGQLPETVVDFVIESIEIPDGVLKGDTELVSFSAAEAGTSVDLRLFEAFNSIAAFELKGSNSNDVAESIKQIQQQAKLTAKYALSV

SEQ ID NO: 4 - DNA, 31 bp, Artificial Sequence
  Forward primer for ywfE
ttttcatatggagagaaaaacagtattggtc

SEQ ID NO: 5 - DNA, 34 bp, Artificial Sequence
  Reverse primer for ywfE
ttttgcggccgctactggcagcacatactttgcc

SEQ ID NO: 6 - DNA, 27 bp, Artificial Sequence
  Forward primer for N107
acaacattcaatgaattattcattgct

SEQ ID NO: 7 - DNA, 27 bp, Artificial Sequence
  Reverse primer for N107F
ttcattgaatgttgtgatggcatccgc

SEQ ID NO: 8 - DNA, 27 bp, Artificial Sequence
  Forward primer for N107L
acaacacttaatgaattattcattgct

SEQ ID NO: 9 - DNA, 27 bp, Artificial Sequence
  Reverse primer for N107L
ttcattaagtgttgtgatggcatccgc

SEQ ID NO: 10 - DNA, 27 bp, Artificial Sequence
  Forward primer for N107I
acaacaattaatgaattattcattgct

SEQ ID NO: 11 - DNA, 27 bp, Artificial Sequence
  ACAACAATTAATGAATTATTCATTGCT
ttcattaattgttgtgatggcatccgc

SEQ ID NO: 12 - DNA, 27 bp, Artificial Sequence
  Forward primer for N107V
acaacagtcaatgaattattcattgct

SEQ ID NO: 13 - DNA, 27 bp, Artificial Sequence
  Reverse primer for N107V
ttcattgactgttgtgatggcatccgc

SEQ ID NO: 14 - DNA, 27 bp, Artificial Sequence
  Forward primer for N107S
acaacatccaatgaattattcattgct

SEQ ID NO: 15 - DNA, 27 bp, Artificial Sequence
  Reverse primer for N107S
ttcattggatgttgtgatggcatccgc

SEQ ID NO: 16 - DNA, 27 bp, Artificial Sequence
  Forward primer for N107P
acaacacccaatgaattattcattgct

SEQ ID NO: 17 - DNA, 27 bp, Artificial Sequence
  Reverse primer for N107P
ttcattgggtgttgtgatggcatccgc

SEQ ID NO: 18 - DNA, 27 bp, Artificial Sequence
  Forward primer for N107T
acaacaaccaatgaattattcattgct

SEQ ID NO: 19 - DNA, 27 bp, Artificial Sequence
  Reverse primer for N107T
ttcattggttgttgtgatggcatccgc

SEQ ID NO: 20 - DNA, 27 bp, Artificial Sequence
  Forward primer for N107A
acaacagccaatgaattattcattgct

SEQ ID NO: 21 - DNA, 27 bp, Artificial Sequence
  Reverse primer for N107A
ttcattggctgttgtgatggcatccgc

SEQ ID NO: 22 - DNA, 27 bp, Artificial Sequence
  Forward primer for N107Y
acaacatacaatgaattattcattgct

SEQ ID NO: 23 - DNA, 27 bp, Artificial Sequence
  Reverse primer for N107Y
ttcattgtatgttgtgatggcatccgc

SEQ ID NO: 24 - DNA, 27 bp, Artificial Sequence
  Forward primer for N107H
acaacacacaatgaattattcattgct

SEQ ID NO: 25 - DNA, 27 bp, Artificial Sequence
  Reverse primer for N107H
ttcattgtgtgttgtgatggcatccgc

SEQ ID NO: 26 - DNA, 26 bp, Artificial Sequence
  Forward primer for N107Q
acaacacagaatgaattattcattgc

SEQ ID NO: 27 - DNA, 27 bp, Artificial Sequence
  ACAACACAGAATGAATTATTCATTGC
ttcattctgtgttgtgatggcatccgc

SEQ ID NO: 28 - DNA, 27 bp, Artificial Sequence
  Forward primer for N107K
acaacaaagaatgaattattcattgct

SEQ ID NO: 29 - DNA, 27 bp, Artificial Sequence
  Reverse primer for N107K
ttcattctttgttgtgatggcatccgc

SEQ ID NO: 30 - DNA, 27 bp, Artificial Sequence
  Forward primer for N107D
acaacagacaatgaattattcattgct

SEQ ID NO: 31 - DNA, 27 bp, Artificial Sequence
  Reverse primer for N107D
ttcattgtctgttgtgatggcatccgc

SEQ ID NO: 32 - DNA, 27 bp, Artificial Sequence
  Forward primer for N107E
acaacagagaatgaattattcattgct

SEQ ID NO: 33 - DNA, 27 bp, Artificial Sequence
  Reverse primer for N107E
ttcattctctgttgtgatggcatccgc

SEQ ID NO: 34 - DNA, 27 bp, Artificial Sequence
  orward primer for N107C
acaacatgtaatgaattattcattgct

SEQ ID NO: 35 - DNA, 27 bp, Artificial Sequence
  Reverse primer for N107C
ttcattacatgttgtgatggcatccgc

SEQ ID NO: 36 - DNA, 27 bp, Artificial Sequence
  Forward primer for N107W
acaacatggaatgaattattcattgct

SEQ ID NO: 37 - DNA, 27 bp, Artificial Sequence
  Reverse primer for N107W
ttcattccatgttgtgatggcatccgc

SEQ ID NO: 38 - DNA, 27 bp, Artificial Sequence
  Forward primer for N107R
acaacaaggaatgaattattcattgct

SEQ ID NO: 39 - DNA, 27 bp, Artificial Sequence
  Reverse primer for N107R
ttcattccttgttgtgatggcatccgc

SEQ ID NO: 40 - DNA, 27 bp, Artificial Sequence
  Forward primer for N107G
acaacagggaatgaattattcattgct

SEQ ID NO: 41 - DNA, 27 bp, Artificial Sequence
  Reverse primer for N107G
ttcattccctgttgtgatggcatccgc

SEQ ID NO: 42 - DNA, 27 bp, Artificial Sequence
  Forward primer for N107
acaacaatgaatgaattattcattgct

SEQ ID NO: 43 - DNA, 27 bp, Artificial Sequence
  Reverse primer for N107M
ttcattcattgttgtgatggcatccgc

SEQ ID NO: 44 - DNA, 27 bp, Artificial Sequence
  Forward primer for N108F
acaaactttgaattattcattgctccg

SEQ ID NO: 45 - DNA, 27 bp, Artificial Sequence
  Reverse primer for N108F
taattcaaagtttgttgtgatggcatc

SEQ ID NO: 46 - DNA, 27 bp, Artificial Sequence
  Forward primer for N108I
acaaacatagaattattcattgctccg

SEQ ID NO: 47 - DNA, 27 bp, Artificial Sequence
  Reverse primer for N108I
taattctatgtttgttgtgatggcatc

SEQ ID NO: 48 - DNA, 27 bp, Artificial Sequence
  Forward primer for N108M
acaaacatggaattattcattgctccg

SEQ ID NO: 49 - DNA, 27 bp, Artificial Sequence
  Reverse primer for N108M
taattccatgtttgttgtgatggcatc

SEQ ID NO: 50 - DNA, 27 bp, Artificial Sequence
  Forward primer for N108V
acaaacgttgaattattcattgctccg

SEQ ID NO: 51 - DNA, 27 bp, Artificial Sequence
  ACAAACGTTGAATTATTCATTGCTCCG
taattcaacgtttgttgtgatggcatc

SEQ ID NO: 52 - DNA, 27 bp, Artificial Sequence
  Forward primer for N108S
acaaactctgaattattcattgctccg

SEQ ID NO: 53 - DNA, 26 bp, Artificial Sequence
  Reverse primer for N108S
taattcagagtttgttgtgatggcat

SEQ ID NO: 54 - DNA, 27 bp, Artificial Sequence
  Forward primer for N108P
acaaaccctgaattattcattgctccg

SEQ ID NO: 55 - DNA, 27 bp, Artificial Sequence
  Reverse primer for N108P
taattcagggtttgttgtgatggcatc

SEQ ID NO: 56 - DNA, 27 bp, Artificial Sequence
  Forward primer for N108T
acaaacactgaattattcattgctccg

SEQ ID NO: 57 - DNA, 27 bp, Artificial Sequence
  Reverse primer for N108T
taattcagtgtttgttgtgatggcatc

SEQ ID NO: 58 - DNA, 27 bp, Artificial Sequence
  Forward primer for N108A
acaaacgctgaattattcattgctccg

SEQ ID NO: 59 - DNA, 27 bp, Artificial Sequence
  Reverse primer for N108A
taattcagcgtttgttgtgatggcatc

SEQ ID NO: 60 - DNA, 27 bp, Artificial Sequence
  Forward primer for N108
acaaactatgaattattcattgctccg

SEQ ID NO: 61 - DNA, 27 bp, Artificial Sequence
  Reverse primer for N108Y
taattcatagtttgttgtgatggcatc

SEQ ID NO: 62 - DNA, 27 bp, Artificial Sequence
  Forward primer for N108H
acaaaccacgaattattcattgctccg

SEQ ID NO: 63 - DNA, 27 bp, Artificial Sequence
  Reverse primer for N108H
taattcgtggtttgttgtgatggcatc

SEQ ID NO: 64 - DNA, 27 bp, Artificial Sequence
  Forward primer for N108Q
acaaaccaagaattattcattgctccg

SEQ ID NO: 65 - DNA, 27 bp, Artificial Sequence
  Reverse primer for N108Q
taattcttggtttgttgtgatggcatc

SEQ ID NO: 66 - DNA, 27 bp, Artificial Sequence
  Forward primer for N108K
acaaacaaagaattattcattgctccg

SEQ ID NO: 67 - DNA, 27 bp, Artificial Sequence
  Reverse primer for N108K
taattctttgtttgttgtgatggcatc

SEQ ID NO: 68 - DNA, 27 bp, Artificial Sequence
  Forward primer for N108D
acaaacgatgaattattcattgctccg

SEQ ID NO: 69 - DNA, 27 bp, Artificial Sequence
  Reverse primer for N108D
taattcatcgtttgttgtgatggcatc

SEQ ID NO: 70 - DNA, 27 bp, Artificial Sequence
  Forward primer for N108E
acaaacgaagaattattcattgctccg

SEQ ID NO: 71 - DNA, 27 bp, Artificial Sequence
  Reverse primer for N108E
taattcttcgtttgttgtgatggcatc

SEQ ID NO: 72 - DNA, 27 bp, Artificial Sequence
  Forward primer for N108C
acaaactgtgaattattcattgctccg

SEQ ID NO: 73 - DNA, 27 bp, Artificial Sequence
  Reverse primer for N108C
taattcacagtttgttgtgatggcatc

SEQ ID NO: 74 - DNA, 27 bp, Artificial Sequence
  Forward primer for N108W
acaaactgggaattattcattgctccg

SEQ ID NO: 75 - DNA, 27 bp, Artificial Sequence
  Reverse primer for N108W
taattcccagtttgttgtgatggcatc

SEQ ID NO: 76 - DNA, 27 bp, Artificial Sequence
  Forward primer for N108R
acaaaccgtgaattattcattgctccg

SEQ ID NO: 77 - DNA, 27 bp, Artificial Sequence
  Reverse primer for N108R
taattcacggtttgttgtgatggcatc

SEQ ID NO: 78 - DNA, 27 bp, Artificial Sequence
  Forward primer for N108G
acaaacggtgaattattcattgctccg

SEQ ID NO: 79 - DNA, 27 bp, Artificial Sequence
  Reverse primer for N108G
taattcaccgtttgttgtgatggcatc

SEQ ID NO: 80 - DNA, 27 bp, Artificial Sequence
  Forward primer for N108L
acaaacttggaattattcattgctccg

SEQ ID NO: 81 - DNA, 27 bp, Artificial Sequence
  Reverse primer for N108L
taattccaagtttgttgtgatggcatc

SEQ ID NO: 82 - DNA, 27 bp, Artificial Sequence
  Forward primer for L110I
aatgaaatattcattgctccgatggcg

SEQ ID NO: 83 - DNA, 27 bp, Artificial Sequence
  Reverse primer for L110I
aatgaatatttcattgtttgttgtgat

SEQ ID NO: 84 - DNA, 27 bp, Artificial Sequence
  Forward primer for L110M
aatgaaatgttcattgctccgatggcg

SEQ ID NO: 85 - DNA, 27 bp, Artificial Sequence
  Reverse primer for L110M
aatgaacatttcattgtttgttgtgat

SEQ ID NO: 86 - DNA, 27 bp, Artificial Sequence
  Forward primer for L110V
aatgaagtgttcattgctccgatggcg

SEQ ID NO: 87 - DNA, 27 bp, Artificial Sequence
  Reverse primer for L110V
aatgaacacttcattgtttgttgtgat

SEQ ID NO: 88 - DNA, 27 bp, Artificial Sequence
  Forward primer for L110S
aatgaaacgttcattgctccgatggcg

SEQ ID NO: 89 - DNA, 27 bp, Artificial Sequence
  AATGAAACGTTCATTGCTCCGATGGCG
aatgaacgtttcattgtttgttgtgat

SEQ ID NO: 90 - DNA, 27 bp, Artificial Sequence
  Forward primer for L110P
aatgaaccgttcattgctccgatggcg

SEQ ID NO: 91 - DNA, 27 bp, Artificial Sequence
  Reverse primer for L110P
aatgaacggttcattgtttgttgtgat

SEQ ID NO: 92 - DNA, 27 bp, Artificial Sequence
  Forward primer for L110T
aatgaaacgttcattgctccgatggcg

SEQ ID NO: 93 - DNA, 27 bp, Artificial Sequence
  Reverse primer for L110T
aatgaacgtttcattgtttgttgtgat

SEQ ID NO: 94 - DNA, 27 bp, Artificial Sequence
  Forward primer for L110A
aatgaagcgttcattgctccgatggcg

SEQ ID NO: 95 - DNA, 27 bp, Artificial Sequence
  Reverse primer for L110A
aatgaacgcttcattgtttgttgtgat

SEQ ID NO: 96 - DNA, 27 bp, Artificial Sequence
  Forward primer for L110Y
aatgaatacttcattgctccgatggcg

SEQ ID NO: 97 - DNA, 27 bp, Artificial Sequence
  Reverse primer for L110Y
aatgaagtattcattgtttgttgtgat

SEQ ID NO: 98 - DNA, 27 bp, Artificial Sequence
  Forward primer for L110H
aatgaacacttcattgctccgatggcg

SEQ ID NO: 99 - DNA, 27 bp, Artificial Sequence
  Reverse primer for L110H
aatgaagtgttcattgtttgttgtgat

SEQ ID NO: 100 - DNA, 27 bp, Artificial Sequence
  Forward primer for L110Q
aatgaacagttcattgctccgatggcg

SEQ ID NO: 101 - DNA, 27 bp, Artificial Sequence
  Reverse primer for L110Q
aatgaactgttcattgtttgttgtgat

SEQ ID NO: 102 - DNA, 27 bp, Artificial Sequence
  Forward primer for L110N
aatgaaaacttcattgctccgatggcg

SEQ ID NO: 103 - DNA, 27 bp, Artificial Sequence
  Reverse primer for L110N
aatgaagttttcattgtttgttgtgat

SEQ ID NO: 104 - DNA, 27 bp, Artificial Sequence
  Forward primer for L110K
aatgaaaagttcattgctccgatggcg

SEQ ID NO: 105 - DNA, 27 bp, Artificial Sequence
  Reverse primer for L110K
aatgaacttttcattgtttgttgtgat

SEQ ID NO: 106 - DNA, 27 bp, Artificial Sequence
  Forward primer for L110D
aatgaagacttcattgctccgatggcg

SEQ ID NO: 107 - DNA, 27 bp, Artificial Sequence
  Reverse primer for L110D
aatgaagtcttcattgtttgttgtgat

SEQ ID NO: 108 - DNA, 27 bp, Artificial Sequence
  Forward primer for L110E
aatgaagaattcattgctccgatggcg

SEQ ID NO: 109 - DNA, 27 bp, Artificial Sequence
  Reverse primer for L110E
aatgaattcttcattgtttgttgtgat

SEQ ID NO: 110 - DNA, 27 bp, Artificial Sequence
  Forward primer for L110C
aatgaatgcttcattgctccgatggcg

SEQ ID NO: 111 - DNA, 27 bp, Artificial Sequence
  Reverse primer for L110C
aatgaagcattcattgtttgttgtgat

SEQ ID NO: 112 - DNA, 27 bp, Artificial Sequence
  Forward primer for L110W
aatgaatggttcattgctccgatggcg

SEQ ID NO: 113 - DNA, 27 bp, Artificial Sequence
  Reverse primer for L110W
aatgaaccattcattgtttgttgtgat

SEQ ID NO: 114 - DNA, 27 bp, Artificial Sequence
  Forward primer for L110R
aatgaacggttcattgctccgatggcg

SEQ ID NO: 115 - DNA, 27 bp, Artificial Sequence
  Reverse primer for L110R
aatgaaccgttcattgtttgttgtgat

SEQ ID NO: 116 - DNA, 27 bp, Artificial Sequence
  Forward primer for L110G
aatgaagggttcattgctccgatggcg

SEQ ID NO: 117 - DNA, 27 bp, Artificial Sequence
  Reverse primer for L110G
aatgaacccttcattgtttgttgtgat

SEQ ID NO: 118 - DNA, 27 bp, Artificial Sequence
  Forward primer for L110F
aatgaattcttcattgctccgatggcg

SEQ ID NO: 119 - DNA, 27 bp, Artificial Sequence
  Reverse primer for L110F
aatgaagaattcattgtttgttgtgat